European Patent Application EP 4 394 037 A1, published July 3, 2024. Title: SITE-SPECIFIC NUCLEASE. Applicant: グランドグリーン株式会社. The sequence listing filed with the application follows.

SEQUENCE LISTING (100 sequences)

SEQ ID NO: 1 - DNA, 50 bp, synthetic construct
  misc_feature 1..50: note = 1
  source 1..50: mol_type = other DNA
gtcaaaagacctttggaatttctactcttgtagatttatgttttggtagt

SEQ ID NO: 2 - DNA, 38 bp, synthetic construct
  misc_feature 1..38: note = 2
  source 1..38: mol_type = other DNA
ccaaaggtcttttgacggtgtttcgtcctttccacaag

SEQ ID NO: 3 - DNA, 44 bp, synthetic construct
  misc_feature 1..44: note = 3
  source 1..44: mol_type = other DNA
ttctactgttgtagatttatgttttggtagtagcgacgtttttt

SEQ ID NO: 4 - DNA, 40 bp, synthetic construct
  misc_feature 1..40: note = 4
  source 1..40: mol_type = other DNA
atctacaacagtagaaattccaaaggtcttttgacggtgt

SEQ ID NO: 5 - DNA, 3789 bp, synthetic construct
  misc_feature 1..3789: note = 5
  source 1..3789: mol_type = other DNA
atgaataacggaactaataacttccaaaacttcatcgggatcagttccttgcagaaaactctccggaatgctctcatcccaactgagactactcagcagttcattgttaagaatggaatcataaaagaggacgagcttaggggggaaaataggcaaatcctcaaggatatcatggatgactattataggggctttatatccgagacactgagcagcattgatgatatagactggacctctcttttcgaaaagatggaaatacaacttaaaaatggagataacaaggacaccctgataaaggaacagaccgaatataggaaggcaattcataaaaagtttgctaacgatgataggtttaaaaacatgttctcagcaaaactcatttcagatatactgcccgaattcgttatccacaacaacaactactccgctagcgaaaaagaggaaaagacccaagtcataaagctgttctctcgattcgcgacgagttttaaagattatttcaagaatcgcgcaaactgtttctcagctgatgatatcagcagctcatcctgtcatcggatcgttaacgataatgctgaaatcttcttctccaatgcacttgtttataggcgcattgttaaatctctctcaaacgatgatatcaataagatttccggcgatatgaaggacagtcttaaggagatgagcctcgaagagatatactcatacgagaaatatggcgaatttatcacccaggaagggatttccttctataatgacatttgcggcaaagtcaattccttcatgaacctgtattgccaaaaaaataaagaaaacaagaacctctataagctgcaaaagttgcataagcaaatactttgtatcgcggatacaagctatgaagttccctacaagttcgagagtgatgaggaggtgtatcaatctgtcaatggtttccttgataatatttcttctaagcatattgttgaacgactccgaaagataggagacaactataatggatacaatttggataaaatctacatcgtgtctaaattttacgagagtgtgtcacaaaaaacatatagagactgggagacaattaataccgccctggagatacattacaacaatatacttcccgggaacgggaagtctaaggcagacaaggtgaagaaagccgtgaagaacgacttgcaaaagtcaattaccgaaatcaatgagcttgtttcaaactataaactttgttcagatgacaatattaaagccgaaacctatattcatgaaatctctcatattctgaataactttgaggcgcaagaactgaaatataacccagaaatacacctcgttgagtccgaactgaaagcaagcgaactgaaaaatgttttggacgtgataatgaacgcttttcattggtgctcagtctttatgacagaggagcttgttgacaaggataacaatttctatgcggaactggaagagatttacgacgaaatctatccggtcatatccctgtataacctggttcgcaactatgtcacgcaaaaaccatacagcacgaagaagattaaactgaactttggtattccgacgctggccgatggatggtcaaaatctaaggaatactcaaacaatgccataatcctgatgcgagataacctctactaccttggaatctttaatgctaaaaataaacccgataaaaaaattatcgaagggaacacgagtgaaaacaaaggtgattataaaaaaatgatatataatctgcttccaggaccaaataagatgatacccaaagttttcctttcttcaaagaccggcgtcgagacatataaaccatccgcgtacatacttgaaggctacaaacaaaataaacatatcaaatcatctaaggattttgacattacgttctgtcatgatttgattgactatttcaaaaattgcatagccattcatccagagtggaaaaactttgggtttgacttctctgataccagtacatatgaagacataagtggattttaccgagaagtagagctccaaggttataaaatagactggacctatatatctgaaaaggatatagaccttttgcaagagaagggacagctttatcttttccaaatctacaacaaagacttcagtaagaaaagtaccgggaatgacaatcttcataccatgtatctgaagaacctgttctccgaagaaaatctgaaggacatagtcctgaagcttaatggcgaagcggaaatttttttccgaaagagctctattaagaaccccataatacataagaagggaagcattctcgttaatcgaacgtatgaggccgaagagaaagatcaatttgggaatatccaaatcgttcgaaagaacataccagaaaatatttaccaagaattgtacaaatattttaacgataaaagcgacaaagaactgtctgatgaagctgctaagctgaaaaacgtcgtcggccatcatgaggccgcgacgaatatagtcaaggattaccgatatacatacgataagtatttcctgcatatgcccatcactatcaactttaaggcaaataagactggattcattaatgacagaatactgcaatacatagctaaagaaaaagatttgcatgttattggcattgacaggggtgagcgcaatcttatctatgtaagcgtcattgatacttgcgggaatatcgtagagcagaagtcatttaatattgtaaatgggtacgattaccaaatcaagttgaagcagcaagagggagcacgacagattgcccgcaaggagtggaaagagatcggaaagataaaggagatcaaggaggggtatttgtcccttgttatacacgaaatttccaagatggtaatcaagtacaacgctataattgctatggaggatctctcctatggatttaaaaagggaagatttaaagtcgagcggcaggtatatcagaaatttgaaacaatgcttattaataaacttaattatctcgttttcaaagacattagtatcaccgaaaacggtgggctgttgaagggctatcaacttacgtacataccagataagcttaagaatgtgggtcaccaatgcggatgcatattctacgtgcccgcagcttatacaagcaaaatcgacccaacaacgggtttcgtaaacatatttaagttcaaggatctcaccgtggatgccaagcgagagttcataaaaaaatttgactcaatcagatatgactcagaaaagaatcttttttgttttaccttcgactacaataatttcattacacaaaatacggttatgagcaagtcatcctggtccgtatatacgtatggagtgcgcataaagcggagattcgttaacgggcgattttctaatgagtccgatacaatcgatataacaaaggatatggaaaaaactctggaaatgactgatataaattggagggacggtcatgacctcaggcaagacattatcgattatgagatcgtgcaacatatttttgagatctttcggttgactgtccaaatgaggaactctctgtctgaattggaagatagggactacgatcgcctgataagccccgtgttgaacgagaataacatattctacgattccgcgaaagccggggatgcgctccctaaggacgccgatgcaaatggggcctattgtattgctttgaaagggctgtacgaaatcaaacagatcaccgaaaactggaaagaagacgggaagtttagtcgggataaactgaagatatccaacaaggactggtttgactttatccaaaataagcgatatttg

SEQ ID NO: 6 - protein, 1263 aa, synthetic construct
  REGION 1..1263: note = 6
MNNGTNNFQNFIGISSLQKTLRNALIPTETTQQFIVKNGIIKEDELRGENRQILKDIMDDYYRGFISETLSSIDDIDWTSLFEKMEIQLKNGDNKDTLIKEQTEYRKAIHKKFANDDRFKNMFSAKLISDILPEFVIHNNNYSASEKEEKTQVIKLFSRFATSFKDYFKNRANCFSADDISSSSCHRIVNDNAEIFFSNALVYRRIVKSLSNDDINKISGDMKDSLKEMSLEEIYSYEKYGEFITQEGISFYNDICGKVNSFMNLYCQKNKENKNLYKLQKLHKQILCIADTSYEVPYKFESDEEVYQSVNGFLDNISSKHIVERLRKIGDNYNGYNLDKIYIVSKFYESVSQKTYRDWETINTALEIHYNNILPGNGKSKADKVKKAVKNDLQKSITEINELVSNYKLCSDDNIKAETYIHEISHILNNFEAQELKYNPEIHLVESELKASELKNVLDVIMNAFHWCSVFMTEELVDKDNNFYAELEEIYDEIYPVISLYNLVRNYVTQKPYSTKKIKLNFGIPTLADGWSKSKEYSNNAIILMRDNLYYLGIFNAKNKPDKKIIEGNTSENKGDYKKMIYNLLPGPNKMIPKVFLSSKTGVETYKPSAYILEGYKQNKHIKSSKDFDITFCHDLIDYFKNCIAIHPEWKNFGFDFSDTSTYEDISGFYREVELQGYKIDWTYISEKDIDLLQEKGQLYLFQIYNKDFSKKSTGNDNLHTMYLKNLFSEENLKDIVLKLNGEAEIFFRKSSIKNPIIHKKGSILVNRTYEAEEKDQFGNIQIVRKNIPENIYQELYKYFNDKSDKELSDEAAKLKNVVGHHEAATNIVKDYRYTYDKYFLHMPITINFKANKTGFINDRILQYIAKEKDLHVIGIDRGERNLIYVSVIDTCGNIVEQKSFNIVNGYDYQIKLKQQEGARQIARKEWKEIGKIKEIKEGYLSLVIHEISKMVIKYNAIIAMEDLSYGFKKGRFKVERQVYQKFETMLINKLNYLVFKDISITENGGLLKGYQLTYIPDKLKNVGHQCGCIFYVPAAYTSKIDPTTGFVNIFKFKDLTVDAKREFIKKFDSIRYDSEKNLFCFTFDYNNFITQNTVMSKSSWSVYTYGVRIKRRFVNGRFSNESDTIDITKDMEKTLEMTDINWRDGHDLRQDIIDYEIVQHIFEIFRLTVQMRNSLSELEDRDYDRLISPVLNENNIFYDSAKAGDALPKDADANGAYCIALKGLYEIKQITENWKEDGKFSRDKLKISNKDWFDFIQNKRYL

SEQ ID NO: 7 - DNA, 66 bp, synthetic construct
  misc_feature 1..66: note = 7
  source 1..66: mol_type = other DNA
gactataaggaccacgacggagactacaaggatcatgatattgattacaaagacgatgacgataag

SEQ ID NO: 8 - protein, 22 aa, synthetic construct
  REGION 1..22: note = 8
DYKDHDGDYKDHDIDYKDDDDK

SEQ ID NO: 9 - DNA, 21 bp, synthetic construct
  misc_feature 1..21: note = 9
  source 1..21: mol_type = other DNA
ccaaagaagaagcggaaggtc

SEQ ID NO: 10 - protein, 7 aa, synthetic construct
  REGION 1..7: note = 10
PKKKRKV

SEQ ID NO: 11 - DNA, 48 bp, synthetic construct
  misc_feature 1..48: note = 11
  source 1..48: mol_type = other DNA
aaaaggccggcggccacgaaaaaggccggccaggcaaaaaagaaaaag

SEQ ID NO: 12 - protein, 16 aa, synthetic construct
  REGION 1..16: note = 12
KRPAATKKAGQAKKKK

SEQ ID NO: 13 - DNA, 90 bp, synthetic construct
  misc_feature 1..90: note = 13
  source 1..90: mol_type = other DNA
tatccttatgatgttcctgattatgctggatatccttatgatgttcctgattatgctggatcttatccttatgatgttcctgattatgct

SEQ ID NO: 14 - protein, 30 aa, synthetic construct
  REGION 1..30: note = 14
YPYDVPDYAGYPYDVPDYAGSYPYDVPDYA

SEQ ID NO: 15 - DNA, 37 bp, synthetic construct
  misc_feature 1..37: note = 15
  source 1..37: mol_type = other DNA
aggctatgaataacggaactaataacttccaaaactt

SEQ ID NO: 16 - DNA, 35 bp, synthetic construct
  misc_feature 1..35: note = 16
  source 1..35: mol_type = other DNA
ccgttattcatagcctgagaccctgataataatta

SEQ ID NO: 17 - DNA, 29 bp, synthetic construct
  misc_feature 1..29: note = 17
  source 1..29: mol_type = other DNA
aggctatgccaaagaagaagcggaaggtc

SEQ ID NO: 18 - DNA, 35 bp, synthetic construct
  misc_feature 1..35: note = 18
  source 1..35: mol_type = other DNA
ttctttggcatagcctgagaccctgataataatta

SEQ ID NO: 19 - DNA, 39 bp, synthetic construct
  misc_feature 1..39: note = 19
  source 1..39: mol_type = other DNA
cggaatgaactcatcccaactgagactactcagcagttc

SEQ ID NO: 20 - DNA, 41 bp, synthetic construct
  misc_feature 1..41: note = 20
  source 1..41: mol_type = other DNA
gatgagttcattccggagagttttctgcaaggaactgatcc

SEQ ID NO: 21 - DNA, 32 bp, synthetic construct
  misc_feature 1..32: note = 21
  source 1..32: mol_type = other DNA
tatttcaggaatcgcgcaaactgtttctcagc

SEQ ID NO: 22 - DNA, 39 bp, synthetic construct
  misc_feature 1..39: note = 22
  source 1..39: mol_type = other DNA
gcgattcctgaaataatctttaaaactcgtcgcgaatcg

SEQ ID NO: 23 - DNA, 39 bp, synthetic construct
  misc_feature 1..39: note = 23
  source 1..39: mol_type = other DNA
gatgataaaagcagctcatcctgtcatcggatcgttaac

SEQ ID NO: 24 - DNA, 35 bp, synthetic construct
  misc_feature 1..35: note = 24
  source 1..35: mol_type = other DNA
gctgcttttatcatcagctgagaaacagtttgcgc

SEQ ID NO: 25 - DNA, 40 bp, synthetic construct
  misc_feature 1..40: note = 25
  source 1..40: mol_type = other DNA
tgtatcagagatacaagctatgaagttccctacaagttcg

SEQ ID NO: 26 - DNA, 42 bp, synthetic construct
  misc_feature 1..42: note = 26
  source 1..42: mol_type = other DNA
tgtatctctgatacaaagtatttgcttatgcaacttttgcag

SEQ ID NO: 27 - DNA, 37 bp, synthetic construct
  misc_feature 1..37: note = 27
  source 1..37: mol_type = other DNA
tggtgcaaagtctttatgacagaggagcttgttgaca

SEQ ID NO: 28 - DNA, 40 bp, synthetic construct
  misc_feature 1..40: note = 28
  source 1..40: mol_type = other DNA
aaagactttgcaccaatgaaaagcgttcattatcacgtcc

SEQ ID NO: 29 - DNA, 37 bp, synthetic construct
  misc_feature 1..37: note = 29
  source 1..37: mol_type = other DNA
tggtgcagagtctttatgacagaggagcttgttgaca

SEQ ID NO: 30 - DNA, 40 bp, synthetic construct
  misc_feature 1..40: note = 30
  source 1..40: mol_type = other DNA
aaagactctgcaccaatgaaaagcgttcattatcacgtcc

SEQ ID NO: 31 - DNA, 39 bp, synthetic construct
  misc_feature 1..39: note = 31
  source 1..39: mol_type = other DNA
aaatctagggaatactcaaacaatgccataatcctgatg

SEQ ID NO: 32 - DNA, 31 bp, synthetic construct
  misc_feature 1..31: note = 32
  source 1..31: mol_type = other DNA
gtattccctagattttgaccatccatcggcc

SEQ ID NO: 33 - DNA, 40 bp, synthetic construct
  misc_feature 1..40: note = 33
  source 1..40: mol_type = other DNA
atatataaactgcttccaggaccaaataagatgataccca

SEQ ID NO: 34 - DNA, 48 bp, synthetic construct
  misc_feature 1..48: note = 34
  source 1..48: mol_type = other DNA
aagcagtttatatatcatttttttataatcacctttgttttcactcgt

SEQ ID NO: 35 - DNA, 40 bp, synthetic construct
  misc_feature 1..40: note = 35
  source 1..40: mol_type = other DNA
atatatagactgcttccaggaccaaataagatgataccca

SEQ ID NO: 36 - DNA, 48 bp, synthetic construct
  misc_feature 1..48: note = 36
  source 1..48: mol_type = other DNA
aagcagtctatatatcatttttttataatcacctttgttttcactcgt

SEQ ID NO: 37 - DNA, 42 bp, synthetic construct
  misc_feature 1..42: note = 37
  source 1..42: mol_type = other DNA
ccaaataggatgatacccaaagttttcctttcttcaaagacc

SEQ ID NO: 38 - DNA, 43 bp, synthetic construct
  misc_feature 1..43: note = 38
  source 1..43: mol_type = other DNA
tatcatcctatttggtcctggaagcagattatatatcattttt

SEQ ID NO: 39 - DNA, 40 bp, synthetic construct
  misc_feature 1..40: note = 39
  source 1..40: mol_type = other DNA
atagccaaacatccagagtggaaaaactttgggtttgact

SEQ ID NO: 40 - DNA, 48 bp, synthetic construct
  misc_feature 1..48: note = 40
  source 1..48: mol_type = other DNA
tggatgtttggctatgcaatttttgaaatagtcaatcaaatcatgaca

SEQ ID NO: 41 - DNA, 40 bp, synthetic construct
  misc_feature 1..40: note = 41
  source 1..40: mol_type = other DNA
atagccagacatccagagtggaaaaactttgggtttgact

SEQ ID NO: 42 - DNA, 48 bp, synthetic construct
  misc_feature 1..48: note = 42
  source 1..48: mol_type = other DNA
tggatgtctggctatgcaatttttgaaatagtcaatcaaatcatgaca

SEQ ID NO: 43 - DNA, 45 bp, synthetic construct
  misc_feature 1..45: note = 43
  source 1..45: mol_type = other DNA
aaaagtaaagggaatgacaatcttcataccatgtatctgaagaac

SEQ ID NO: 44 - DNA, 45 bp, synthetic construct
  misc_feature 1..45: note = 44
  source 1..45: mol_type = other DNA
attccctttacttttcttactgaagtctttgttgtagatttggaa

SEQ ID NO: 45 - DNA, 45 bp, synthetic construct
  misc_feature 1..45: note = 45
  source 1..45: mol_type = other DNA
aaaagtagagggaatgacaatcttcataccatgtatctgaagaac

SEQ ID NO: 46 - DNA, 45 bp, synthetic construct
  misc_feature 1..45: note = 46
  source 1..45: mol_type = other DNA
attccctctacttttcttactgaagtctttgttgtagatttggaa

SEQ ID NO: 47 - DNA, 49 bp, synthetic construct
  misc_feature 1..49: note = 47
  source 1..49: mol_type = other DNA
gcgacggatatagtcaaggattaccgatatacatacgataagtatttcc

SEQ ID NO: 48 - DNA, 32 bp, synthetic construct
  misc_feature 1..32: note = 48
  source 1..32: mol_type = other DNA
gactatatccgtcgcggcctcatgatggccga

SEQ ID NO: 49 - DNA, 43 bp, synthetic construct
  misc_feature 1..43: note = 49
  source 1..43: mol_type = other DNA
aaggataaacgatatacatacgataagtatttcctgcatatgc

SEQ ID NO: 50 - DNA, 35 bp, synthetic construct
  misc_feature 1..35: note = 50
  source 1..35: mol_type = other DNA
atatcgtttatccttgactatattcgtcgcggcct

SEQ ID NO: 51 - DNA, 43 bp, synthetic construct
  misc_feature 1..43: note = 51
  source 1..43: mol_type = other DNA
aaggatagacgatatacatacgataagtatttcctgcatatgc

SEQ ID NO: 52 - DNA, 35 bp, synthetic construct
  misc_feature 1..35: note = 52
  source 1..35: mol_type = other DNA
atatcgtctatccttgactatattcgtcgcggcct

SEQ ID NO: 53 - DNA, 35 bp, synthetic construct
  misc_feature 1..35: note = 53
  source 1..35: mol_type = other DNA
tttaaaagaggaagatttaaagtcgagcggcaggt

SEQ ID NO: 54 - DNA, 39 bp, synthetic construct
  misc_feature 1..39: note = 54
  source 1..39: mol_type = other DNA
tcttcctcttttaaatccataggagagatcctccatagc

SEQ ID NO: 55 - DNA, 36 bp, synthetic construct
  misc_feature 1..36: note = 55
  source 1..36: mol_type = other DNA
gtgggtaaacaatgcggatgcatattctacgtgccc

SEQ ID NO: 56 - DNA, 46 bp, synthetic construct
  misc_feature 1..46: note = 56
  source 1..46: mol_type = other DNA
gcattgtttacccacattcttaagcttatctggtatgtacgtaagt

SEQ ID NO: 57 - DNA, 36 bp, synthetic construct
  misc_feature 1..36: note = 57
  source 1..36: mol_type = other DNA
gtgggtagacaatgcggatgcatattctacgtgccc

SEQ ID NO: 58 - DNA, 46 bp, synthetic construct
  misc_feature 1..46: note = 58
  source 1..46: mol_type = other DNA
gcattgtctacccacattcttaagcttatctggtatgtacgtaagt

SEQ ID NO: 59 - DNA, 37 bp, synthetic construct
  misc_feature 1..37: note = 59
  source 1..37: mol_type = other DNA
aggaacgctctgtctgaattggaagatagggactacg

SEQ ID NO: 60 - DNA, 33 bp, synthetic construct
  misc_feature 1..33: note = 60
  source 1..33: mol_type = other DNA
agacagagcgttcctcatttggacagtcaaccg

SEQ ID NO: 61 - DNA, 40 bp, synthetic construct
  misc_feature 1..40: note = 61
  source 1..40: mol_type = other DNA
gcctataatattgctttgaaagggctgtacgaaatcaaac

SEQ ID NO: 62 - DNA, 33 bp, synthetic construct
  misc_feature 1..33: note = 62
  source 1..33: mol_type = other DNA
agcaatattataggccccatttgcatcggcgtc

SEQ ID NO: 63 - DNA, 873 bp, synthetic construct
  misc_feature 1..873: note = 63
  source 1..873: mol_type = other DNA
atgagtaaatcatggggtaagttcattgaagaggaagaagcagagatggctagcagacgtaacctcatgatagttgacggaactaatctagggtttcggttcaaacacaataacagcaagaaaccctttgcttcctcgtatgtttcaaccattcagagtctagccaaatcctattccgctagaaccactatagttcttggcgataaggggaagtctgtctttcgtttagagcatcttcctgaatacaaaggcaatagagatgagaagtatgcccaaaggacagaggaggaaaaggcgttagatgagcaattcttcgaatatctcaaagacgcttttgagttgtgcaagacaacgtttccaactttcactatcagaggagtcgaagcagatgatatggctgcgtacatcgttaaactcattggtcatttgtacgatcatgtgtggttgatttctacagacggagattgggatacacttttaactgataaggtgtctaggttctcatttacgaccagacgagagtatcacttgagagatatgtacgaacatcacaatgttgacgatgtagaacagtttatcagcttgaaagccattatgggagatcttggtgacaacatacgtggtgtagaagggattggagcaaaacgaggttacaacatcatcagggaattcggcaatgtgctagacatcattgatcagctgccattgcctggtaagcaaaagtacattcagaatcttaacgcttcggaagagttactcttcagaaaccttatactcgttgatcttccgacgtattgtgtggatgctattgcagctgttggacaagatgtcctggacaagtttaccaaagacatcctggaaatagcggaacaa

SEQ ID NO: 64 - protein, 291 aa, synthetic construct
  REGION 1..291: note = 64
MSKSWGKFIEEEEAEMASRRNLMIVDGTNLGFRFKHNNSKKPFASSYVSTIQSLAKSYSARTTIVLGDKGKSVFRLEHLPEYKGNRDEKYAQRTEEEKALDEQFFEYLKDAFELCKTTFPTFTIRGVEADDMAAYIVKLIGHLYDHVWLISTDGDWDTLLTDKVSRFSFTTRREYHLRDMYEHHNVDDVEQFISLKAIMGDLGDNIRGVEGIGAKRGYNIIREFGNVLDIIDQLPLPGKQKYIQNLNASEELLFRNLILVDLPTYCVDAIAAVGQDVLDKFTKDILEIAEQ

SEQ ID NO: 65 - protein, 276 aa, synthetic construct
  REGION 1..276: note = 65
MATTIANLGSPAPIGNLLIVDGLNVAFRWKHQNILDFKYDYIRTIESLAKSYKAGTIIVCADGGSSYRKEIYPEYKANRKERFADQTKQEAKEFEMFMAEFQDTLTLIKEKYPVFHFRGVEADDIAAYITQSVNYDDCWLISSDKDWDLLISDKVSRFSTVTRKETTVHNWDEHYDFEIDDYITFKCLTGDKGDNVPGVPGVGPKRAVQLMEQYGSIFDIYDACPLEGKYKYIQAVNENAEQLLQNVELMDLITYNEDAIGQENIKVIDNTLGKIL

SEQ ID NO: 66 - protein, 278 aa, synthetic construct
  REGION 1..278: note = 66
MKTFKQFELTNKTLMIVDALNLAFRYKHSKAKDFAEDYLHTVESLAKSYRAQNVIIAADQGSSSYRKTIYANYKQNRKDKYEQQTEAEKLEFELFFEDFSKTLELLTEYYPVLKFQGVEADDIAAYIVAKQHRLQIDQIWLISSDKDWDLLIKPNTSRFSYITRKEITWENWTDHYTFEPEQYIHIKCLIGDSGDNVPGVAGVGPKRAQQLIEEYGTTWDIINSIPISGKYKYIEAINQSKTQLMLNYQLMDLVTYCSDAIGTENCKQIDETLKLCLK

SEQ ID NO: 67 - protein, 290 aa, synthetic construct
  REGION 1..290: note = 67
MKRWSGLVASFKERIMEPNKNALIVDGMNLAFRWKHQGKLDFKQDYINTVKSLAQSYDCSKIIIAGDQGSSAYRKFIDPQYKANRAEKYKDQTEQEKEDIKLFFEEYERTLEGLEEQFLLLRYANVEADDLVAYVVSKREEMGIEDIWMISSDRDWDLLVNENVSRFSTVTRKETTVFNWEEFFDFPQEDYISFKVLTGDKGDNIDGVAGIGPKRATELIKEYGTAFDIYDAIPIPSRYKYIQALNASKELILKNYRMMDLVSYCAEAIEHPGHSLLEIDERVKEYINVN

SEQ ID NO: 68 - protein, 287 aa, synthetic construct
  REGION 1..287: note = 68
  SITE 36: note = misc_feature - Xaa can be any naturally occurring amino acid
  SITE 71: note = misc_feature - Xaa can be any naturally occurring amino acid
  SITE 74: note = misc_feature - Xaa can be any naturally occurring amino acid
  SITE 81: note = misc_feature - Xaa can be any naturally occurring amino acid
  SITE 101: note = misc_feature - Xaa can be any naturally occurring amino acid
  SITE 107: note = misc_feature - Xaa can be any naturally occurring amino acid
  SITE 119: note = misc_feature - Xaa can be any naturally occurring amino acid
  REGION 122..123: note = misc_feature - Xaa can be any naturally occurring amino acid
  SITE 125: note = misc_feature - Xaa can be any naturally occurring amino acid
  REGION 133..134: note = misc_feature - Xaa can be any naturally occurring amino acid
  SITE 136: note = misc_feature - Xaa can be any naturally occurring amino acid
  SITE 194: note = misc_feature - Xaa can be any naturally occurring amino acid
MAINFSSLGNQIQNGNLLIVDGLNVAFRWKHSKQLXFKHDYVRTVESLAKSYNCGNIIVLADGGSTYRKNXSPXYKANRKXKYAEQTEQEKAEFAQFMGEXSNAFTXLKKKGHLTIKQXGLXXDXLAAWIVGXXKXFGIDEIWLISSDKDWDLLIQDKVSRFSTVTRKEITLDNWEDHYDVEPDKYLTLKCLAXDTGDNVPGIAGIGPKRAVSLIEQYGDLFDIYNACPIDSKYKFIQTLNENADRLLLNAELMDLESYSEQAIIEADMNIEDLFSQILEYLNEVRD

SEQ ID NO: 69 - protein, 315 aa, synthetic construct
  REGION 1..315: note = 69
MTNYSLIDGNSLGHFYNNAKPLMIGEVQVQAIYGTLKRLRAHCAGFQDYQPVVLWDGASWRKMMFAEYKENRDRKETKNEIRMQEMKASYKKQAPYLKKALRFLGIPQVSALNMEADDLGAILTDRYTKNGSKIILLTGDKDWLQLVGPGVVWKDFANDRLVTQKNFAEFTGVEDVRKFVEVKALCGDQGDNVAGVGGIGEKGAIEFINTYGSVANFTNGVILDKTIDLKGVPKKYRNLVEDEDKAITFKRNIDLVDLRTTARPAPLALEVDKGTADADKFRQFCELLLFKSFTKDFDEWISVFPAFRAPRALAA

SEQ ID NO: 70 - protein, 290 aa, synthetic construct
  REGION 1..290: note = 70
MSKSWGQMKAEADEKLASRKNLMIVDGTNLGFRFKKDIVKPIASSFLNTINSLANSYDAKDTIILGDKGKSIFRTEIYPEYKGNRDERFSQRTEEEVAADKLFFEYLEEAFDLASSTYPTFKIRGVEADDMAGFIIQLIGGEYDHVWLISTDGDWDTLLSPTVSRFSFTTRREYHERDMYENHQCDTVEQFASLKALMGDMGDNIRGVEGLGPKRGYGLLREYGTALDILDALPLPGKQKFIQNLNASAELIERNLQLVDLPTFCGEAIAAAGQDVYNKFKEDILKVAHK

SEQ ID NO: 71 - protein, 293 aa, synthetic construct
  REGION 1..293: note = 71
MSTKSWKQIRDEEVAEFESRNNLVVIDLVNIAHRVSQNIKDGKAFARKLLEDIKRFEKEYHGRKVIVLTDKGKSSYRVALFPEYKDNRRKAREKRSEAEQRAQREWFSKLKEGIRIVEETIKIFGYEGVEADDMAAVIVDQYSGTQLFDHIWLISTDGDWDLLLKDDVSRYSFYTQREYKLKDMYENSGVDTPEQLASLKALQGDRKDNIDGVEGVGTKRGYGLIREFGSALDIVEAIPLPGKQAFIRKVNESAELIERNVQLVDLVSFSAEALAHAGVYNKFVEELEEIINA

SEQ ID NO: 72 - protein, 292 aa, synthetic construct
  REGION 1..292: note = 72
MTKGWKASQAEYKEELASRNNLMIVDGLNLGFRFQGQVKKPFASNYLNTVQSFAKSYSARDTIILSDKGVSTFRKNIHEGYKGQRAERNKNKTEEEKEQTRLFFEYFEEAYELASTVFPCFRYRGVEADDMAGVIVALAIMYGNYDTIWLISTDGDWDTLLQATVKRFSYKTRREYTVESMYEEHGVDTVEQFISLKAIMGDPGDSINGVDGIGAKRGYSIIREYGSVMDIIDSMPLPGKQQFIKNLNNSEDLLLRNIQLVDLPSFSAEALEAAGVYKEFYEQIKEIVSAKA

SEQ ID NO: 73 - protein, 292 aa, synthetic construct
  REGION 1..292: note = 73
MSKSWGTMKREAEQRLASRRNLMIVDGTNLGFRFKKDSGKPIAASFANTINSLANSYDAKHTIVLGDKGKSIFRTNIFPEYKGNRDAKYADRSAAEVEADRQFFEYLDDAFDLIASQFPTFRIRGVEADDMAAFIIQLIGHHYDHIWLISTDGDWDTLLAPNISRFSFTTRKEYHEKDMFDNHNVDTVDQFISLKAIMGDMGDNIRGVEGIGEKRGYNLIREHGSVLDIIDALPLPGTQKFVQALNKSGELMERNLTLVDLPSFCGEAVAAAGQDIYDQFVKDIMAVATGEV

SEQ ID NO: 74 - protein, 288 aa, synthetic construct
  REGION 1..288: note = 74
MSSWTKMLSTELVGDNLLIVDMMNFSRSISSASSVEDFAKKLETSIRSFAKSYSCGKVVLLSDKGVSSYRKEILPEYKENRKKKREAMSEAQRAAEAEWFFMMRDAVDSLADTFPLFKYQDVEADDMAALITDWAIDGEHVEEVFLLSTDGDWDTFLRERVSRFAFTTRKMFTIDNMFEEHGADSPEQFALLKAIQGDLGDNIRGIDGVGKKRGYSVIREFNSTAHFLDSIPDLVGSQKFICNIRDGQDIIERNLLLVDLRSFAYDALVHAGVYDEFKSRVYSEVFGE

SEQ ID NO: 75 - protein, 288 aa, synthetic construct
  REGION 1..288: note = 75
MAEEAEAEVKARRNLVIIDGTNLAFRFNGNKGESFSTSYTKTINSFAKSYSARHTIVLGDKGKSIFRTEIDPEYKANRDAKYDSQSEQEKEESRAFFECVAEAFELCAAILPTIRIRGIEADDIAAYIKARIGHLYDHIWLISTDGDWDILLDEKTSRFSFQTRKEYRIETMYDHHGVDTVDQFISLKAIMGDTGDNIIGVEGIGIKRGYNIIKEYGSALDIIDQIPLPGKQKFIQNLNASGDLIMRNLSLVDLNSFCVDAIMAVGQDAMDSINKVLDTLAEEITNGN

SEQ ID NO: 76 - protein, 290 aa, synthetic construct
  REGION 1..290: note = 76
MMDMWNMATEEAMMPKNNLLIVDGLNLAFRYKHRGTTDFAADYVKTVNSLAKSYHAREIVILVDYKGSWFRKDLHPKYKFDRKAKFADQTEEEKLAAEQFFEDFNKAIELCECNFHVIKLEGVEADDTAAYLVEEFEDTDDFDHIWLISTDKDWDELLGEKVSRFSYTTRKEYNLDNFYEYHQCDTPDEYTSIKAIMGDPGDSVYGVNGIGAKRAYNLVRQYGDALEIATQLPIEGKQKYIEELNKSEEKLILNTQLVDLRSFHKEAIAFPSPENLLYLEQVCNNLRGAA

SEQ ID NO: 77 - protein, 255 aa, synthetic construct
  REGION 1..255: note = 77
MIRTVESLAKSYSALHIVCAWDHRSSSYRKSIYPGYKGGRKEKYKDQTPEEKLQAEMFFNGLDEAYQHMVIHEKNTGFVTNFKFEFVEADDPIALTVQVMEPFVDHIWVISTDQDFCQLISNKVSLFAYKSRKEFTLDTMFEYTNADSGEQHLFIKCLQGDSGDSVPGVPDVGPKRGYGLAREYGDIFSLIAALPIEGKQKYIVKLNEFGASNLMLNLELMDLKSYCATAIAFPNPANLDYMFDKLEKIKEIYNV

SEQ ID NO: 78 - protein, 321 aa, synthetic construct
  REGION 1..321: note = 78
MKRYLLIDGNNIAHAANGTKNKLTVGSVETTAIFGFLRQLRKQISIYGQFTPIVLWDGASWRKMQYKDYKENREKNDTAAAQKQKAERESTKKQIPAIQKALQLLGVTQIKAANMEADDLAAICADRYIKQGAGVVLVSGDKDWLQLVGPNCMWFDPINDRKVRTVADLADEKNKLGIAVKSFKQFVEMKALMGDTGDNIPGVGGIGDKGAMEFLAEFESYSNFSNMCLTGEVDLKKLPKKFRDLAESEDKRILFMRNLMLMDLRHPARPAPINLKVDPGSPSIETFTLFCQRLVFKSFLTDIENWVSVFPPFKYREAAAA

SEQ ID NO: 79 - protein, 318 aa, synthetic construct
  REGION 1..318: note = 79
MQRYLLIDGMNIAHAANNAKPLKVGETQVQAIYHFVKIVRKLIATYPTAKPAVLWDGASWRYMDFPDYKSNRKKQDTPSAVKAAEMKKIAEGQIPAIKKAMQLLGVPQVRASNMEADDLAAIMGDRYAAKGGKVVLVSGDKDWVQLVNPNIIWLDPIQDRKIMKAADMLPALGYDLESFEAFVEMKCLWGDEGDGISGVGGIGDKGAIAFLKEYVSVSNFSNMLIDKTLDPKTVPKKFRDFGESEEKQMIYQRNLKLMDLRTKLRPEPVNLRVDTGTPDIERFKTFCNRLMFRSITKDLEPWISVFPAFHHLQEELAA

SEQ ID NO: 80 - DNA, 459 bp, synthetic construct
  misc_feature 1..459: note = CmYLCV promoter
  source 1..459: mol_type = other DNA
tggcagacatactgtcccacaaatgaagatggaatctgtaaaagaaaacgcgtgaaataatgcgtctgacaaaggttaggtcggctgcctttaatcaataccaaagtggtccctaccacgatggaaaaactgtgcagtcggtttggctttttctgacgaacaaataagattcgtggccgacaggtgggggtccaccatgtgaaggcatcttcagactccaataatggagcaatgacgtaagggcttacgaaataagtaagggtagtttgggaaatgtccactcacccgtcagtctataaatacttagcccctccctcattgttaagggagcaaaatctcagagagatagtcctagagagagaaagagagcaagtagcctagaagtagtcaaggcggcgaagtattcaggcaggtggccaggaagaagaaaagccaagacgacgaaaacaggtaagagct

SEQ ID NO: 81 - DNA, 181 bp, synthetic construct
  misc_feature 1..181: note = dMac3
  source 1..181: mol_type = other DNA
atgctccacaaagacgcactacagaagactaaagagagctttttcataccaaagaagtacaacaaagatttgctcctcattttctgaatcctgggactctctagcctgtagaagaagaaaggcaggaatttcagctcaagagaacagatcacaatatttacccacggcactgtctcgcaat

SEQ ID NO: 82 - DNA, 211 bp, synthetic construct
  misc_feature 1..211: note = CaMV 35S terminator
  source 1..211: mol_type = other DNA
gtccgcaaaaatcaccagtctctctctacaaatctatctctctctatttttctccagaataatgtgtgagtagttcccagataagggaattagggttcttatagggtttcgctcatgtgttgagcatataagaaacccttagtatgtatttgtatttgtaaaatacttctatcaataaaatttctaattcctaaaaccaaaatccagtgac

SEQ ID NO: 83 - DNA, 1038 bp, synthetic construct
  misc_feature 1..1038: note = NbACT3 terminator
  source 1..1038: mol_type = other DNA
atacagcattcccagaaagagaaacagaagaaatatacaaactttcattttgagagcagcacctcgtctattgattgcagataatatgcttctcatttgtatttccttttgattatttttgtttctatccctttgtttgagtcaatctcaaatattcggtcattgttggtatgaaaaatcaagcagttcatgttaagagtcaatttaaaattaatatttttatatagagttgtatgtgaaatgatgttgtgatttggtatatatggataaagagcttgtcagttcattttggtgtcatttttttggtatccaaataagaaacacaaaagggatatgtccctctactatcaaatattagttataagtattcatgttatactattcgatattttctaccccaatcgttacctatttaaaagtatttacccctccatctatcaaacccctggacccagctttcctattacatgtggcttcatcttaagcccccaaacctttttcttatttttgatttttaaaggctcatcttaaaatttattactcaaattaatacctcttaataacccacctcaaggacccagtaattaaatatccaattagctccagtaattggggttcatattagctccagtcttaaattttaaaggcgatgatcgtattcctccacttggttcatttatactcaaagaatactcaatgtctttagtgtttagataactttttgtaaatcatatagattgttttaacaaaaaacaattcaatagtagattttcacatgaaagttacataaaaattctttaaaattactttctcaaaaaattgttccaaacatattatcccacaattaaactcaatctgtttttcgaaacctaaatcaaaaccaatccaactaccttatataatatataatcaatacattgtaaagaactgcatgttcttttaaattttgggggcaaagttattccgtacgttcacacatgtactaataggaggtaataaatgatatgtgaaacaatcgaggtgtaaacaagctagcat

SEQ ID NO: 84 - DNA, 1169 bp, synthetic construct
  misc_feature 1..1169: note = Rb7 MAR
  source 1..1169: mol_type = other DNA
tcgattaaaaatcccaattatatttggtctaatttagtttggtattgagtaaaacaaattcgaaccaaaccaaaatataaatatatagtttttatatatatgcctttaagactttttatagaattttctttaaaaaatatctagaaatatttgcgactcttctggcatgtaatatttcgttaaatatgaagtgctccatttttattaactttaaataattggttgtacgatcactttcttatcaagtgttactaaaatgcgtcaatctctttgttcttccatattcatatgtcaaaatctatcaaaattcttatatatctttttcgaatttgaagtgaaatttcgataatttaaaattaaatagaacatatcattatttaggtatcatattgatttttatacttaattactaaatttggttaactttgaaagtgtacatcaacgaaaaattagtcaaacgactaaaataaataaatatcatgtgttattaagaaaattctcctataagaatattttaatagatcatatgtttgtaaaaaaaattaatttttactaacacatatatttacttatcaaaaatttgacaaagtaagattaaaataatattcatctaacaaaaaaaaaaccagaaaatgctgaaaacccggcaaaaccgaaccaatccaaaccgatatagttggtttggtttgattttgatataaaccgaaccaactcggtccatttgcacccctaatcataatagctttaatatttcaagatattattaagttaacgttgtcaatatcctggaaattttgcaaaatgaatcaagcctatatggctgtaatatgaatttaaaagcagctcgatgtggtggtaatatgtaatttacttgattctaaaaaaatatcccaagtattaataatttctgctaggaagaaggttagctacgatttacagcaaagccagaatacaaagaaccataaagtgattgaagctcgaaatatacgaaggaacaaatatttttaaaaaaatacgcaatgacttggaacaaaagaaagtgatatattttttgttcttaaacaagcatcccctctaaagaatggcagttttcctttgcatgtaactattatgctcccttcgttacaaaaattttggactactattgggaacttcttctgaaaatagtg

SEQ ID NO: 85 - DNA, 864 bp, synthetic construct
  misc_feature 1..864: note = CaMV 35S promoter
  source 1..864: mol_type = other DNA
ccgatccattcggtccccagattagccttttcaatttcagaaagaatgctaacccacagatggttagagaggcttacgcagcacgtctcatcaagacgatctacccgagcaataatctccaggaaatcaaataccttcccaagaaggttaaagatgcagtcaaaagattcaggactaactgcatcaagaacacagagaaagatatatttctcaagatcagaagtactattccagtatggacgattcaaggcttgcttcacaaaccaaggcaagtaatagagattggagtctctaaaaaggtagttcccactgaatcaaaggccatggagtcaaagattcaaatagaggacctaacagaactcgccgtaaagactggcgaacagttcatacagagtctcttacgactcaatgacaagaagaaaatcttcgtcaacatggtggagcacgacacacttgtctactccaaaaatatcaaagatacagtctcagaagaccaaagggcaattgagacttttcaacaaagggtaatatccggaaacctcctcggattccattgcccagctatctgtcactttattgtgaagatagtggaaaaggaaggtggctcctacaaatgccatcattgcgataaaggaaaggccatcgttgaagatgcctctgccgacagtggtcccaaagatggacccccacccacgaggagcatcgtggaaaaagaagacgttccaaccacgtcttcaaagcaagtggattgatgtgatatctccactgacgtaagggatgacgcacaatcccactatccttcgcaagacccttcctctatataaggaagttcatttcatttggagagaacacgggggacgagct

SEQ ID NO: 86 - DNA, 43 bp, synthetic construct
  misc_feature 1..43: note = HH ribozyme
  source 1..43: mol_type = other DNA
aaattactgatgagtccgtgaggacgaaacgagtaagctcgtc

SEQ ID NO: 87 - DNA, 20 bp, synthetic construct
  misc_feature 1..20: note = direct repeat
  source 1..20: mol_type = other DNA
taatttctactgttgtagat

SEQ ID NO: 88 - DNA, 20 bp, synthetic construct
  misc_feature 1..20: note = spacer
  source 1..20: mol_type = other DNA
tatgtaggtgtatttggaat

SEQ ID NO: 89 - DNA, 68 bp, synthetic construct
  misc_feature 1..68: note = HDV ribozyme
  source 1..68: mol_type = other DNA
ggccggcatggtcccagcctcctcgctggcgccggctgggcaacatgcttcggcatggcgaatgggac

SEQ ID NO: 90 - DNA, 299 bp, synthetic construct
  misc_feature 1..299: note = Nos terminator
  source 1..299: mol_type = other DNA
agcggccgcccggctgcagatcgttcaaacatttggcaataaagtttcttaagattgaatcctgttgccggtcttgcgatgattatcatataatttctgttgaattacgttaagcatgtaataattaacatgtaatgcatgacgttatttatgagatgggtttttatgattagagtcccgcaattatacatttaatacgcgatagaaaacaaaatatagcgcgcaaactaggataaattatcgcgcgcggtgtcatctatgttactagatccgatgataagctgtcaaacatgagaatt

SEQ ID NO: 91 - protein, 57 aa, synthetic construct
KRPAATKKAGQAKKKKGSYPYDVPDYAGYPYDVPDYAGSYPYDVPDYAGSPKKKRKV

SEQ ID NO: 92 - protein, 62 aa, synthetic construct
KRKNSATVHLCPVPRKRGSYPYDVPDYAGYPYDVPDYAGSYPYDVPDYAGSAAAKRSWSMAF

SEQ ID NO: 93 - protein, 60 aa, synthetic construct
KRKNSATVHLCPVPRKRGSYPYDVPDYAGYPYDVPDYAGSYPYDVPDYAGSRAAKRPRTT

SEQ ID NO: 94 - protein, 77 aa, synthetic construct
KRPAATKKAGQAKKKKGSYPYDVPDYAYPYDVPDYAYPYDVPDYAPAAKRVKLDGGSGGGPAAKRVKLDLEHHHHHH

SEQ ID NO: 95 - protein, 80 aa, synthetic construct
KRPAATKKAGQAKKKKGSYPYDVPDYAGYPYDVPDYAGSYPYDVPDYAGSPKKKRKVGGSGGGPAAKRVKLDLEHHHHHH

SEQ ID NO: 96 - protein, 82 aa, synthetic construct
KRKNSATVHLCPVPRKRGSYPYDVPDYAYPYDVPDYAYPYDVPDYAAAAKRSWSMAFGGSGGGAAAKRSWSMAFLEHHHHHH

SEQ ID NO: 97 - protein, 80 aa, synthetic construct
KRKNSATVHLCPVPRKRGSYPYDVPDYAYPYDVPDYAYPYDVPDYARAAKRPRTTGGSGGGAAAKRSWSMAFLEHHHHHH

SEQ ID NO: 98 - protein, 78 aa, synthetic construct
KRKNSATVHLCPVPRKRGSYPYDVPDYAYPYDVPDYAYPYDVPDYARAAKRPRTTGGSGGGRAAKRPRTTLEHHHHHH

SEQ ID NO: 99 - protein, 72 aa, synthetic construct
KRKNSATVHLCPVPRKRGSYPYDVPDYAYPYDVPDYAYPYDVPDYARAAKRPRTTGGSGGGAAAKRSWSMAF

SEQ ID NO: 100 - protein, 70 aa, synthetic construct
KRKNSATVHLCPVPRKRGSYPYDVPDYAYPYDVPDYAYPYDVPDYARAAKRPRTTGGSGGGRAAKRPRTT